European Patent Application EP 4 737 476 A1, published May 6, 2026. Title: T-CELL RECEPTOR VARIANT AGAINST mKRAS 7-16 G12D. Applicant: Medigene Immunotherapies GmbH. Application EP. The sequence listing filed with the application follows.

SEQUENCE LISTING (48 sequences)

SEQ ID NO: 1 - protein, 10 aa, synthetic construct
VVVGADGVGK

SEQ ID NO: 2 - protein, 5 aa, synthetic construct
WNHNN

SEQ ID NO: 3 - protein, 6 aa, synthetic construct
SYGVHD

SEQ ID NO: 4 - protein, 14 aa, synthetic construct
CASSGAGETGELFF

SEQ ID NO: 5 - DNA, 15 bp, synthetic construct
  source 1..15: mol_type = other DNA
tggaaccacaacaac

SEQ ID NO: 6 - DNA, 18 bp, synthetic construct
  source 1..18: mol_type = other DNA
tcttacggcgtgcacgac

SEQ ID NO: 7 - DNA, 42 bp, synthetic construct
  source 1..42: mol_type = other DNA
tgtgcctctagcggagccggcgaaaccggcgaactgtttttc

SEQ ID NO: 8 - protein, 132 aa, synthetic construct
MGTRLFFYVALCLLWAGHRDAEITQSPRHKITETGRQVTLACHQTWNHNNMFWYRQDLGHGLRLIHYSYGVHDTNKGEVSDGYSVSRSNTEDLPLTLESAASSQTSVYFCASSGAGETGELFFGEGSRLTVL

SEQ ID NO: 9 - DNA, 396 bp, synthetic construct
  source 1..396: mol_type = other DNA
atgggcaccagactgttcttttacgtggccctgtgcctgctgtgggccggacatagagatgccgagatcacacagagccccagacacaagatcaccgagacaggcagacaagtgaccctggcctgtcaccagacctggaaccacaacaacatgttctggtacagacaggacctcggccacggcctgagactgatccactactcttacggcgtgcacgacaccaacaagggcgaagtgtctgacggctacagcgtgtccagaagcaacaccgaggacctgcctctgacactggaatctgccgccagctctcagaccagcgtgtacttttgtgcctctagcggagccggcgaaaccggcgaactgtttttcggagagggcagcagactgaccgtgctc

SEQ ID NO: 10 - protein, 177 aa, synthetic construct
EDLNKVFPPEVAVFEPSKAEIAHTQKATLVCLATGFFPDHVELSWWVNGKEVHSGVSTDPQPLKEQPALNDSRYCLSSRLRVSATFWQNPRNHFRCQVQFYGLSENDEWTQDRAKPVTQIVSAEAWGRADCGITSASYHQGVLSATILYEILLGKATLYAVLVSALVLMAMVKRKDF

SEQ ID NO: 11 - DNA, 531 bp, synthetic construct
  source 1..531: mol_type = other DNA
gaggacctgaacaaggtgttccctccggaggtggccgtgttcgagcccagcaaagccgagatcgcgcacacccagaaggccaccctggtgtgcctggccaccggcttcttccccgaccacgtggagctgagctggtgggtgaacggcaaggaggtgcacagcggcgtgagcaccgacccccagcccctgaaggagcagcccgccctgaacgacagccgctactgcctgagcagccgcctgcgcgtgagcgccaccttctggcagaacccccgcaaccacttccgctgccaggtgcagttctacggcctgagcgagaacgacgagtggacccaggaccgcgccaagcccgtgacccagatcgtgagcgccgaggcctggggccgcgccgactgcggcattaccagcgcgagctaccatcagggcgtgctgagcgccaccatcctgtacgagatcctgctgggcaaggccaccctgtacgccgtgctggtgagcgccctggtgctgatggcgatggtgaagcgcaaggacttc

SEQ ID NO: 12 - protein, 309 aa, synthetic construct
MGTRLFFYVALCLLWAGHRDAEITQSPRHKITETGRQVTLACHQTWNHNNMFWYRQDLGHGLRLIHYSYGVHDTNKGEVSDGYSVSRSNTEDLPLTLESAASSQTSVYFCASSGAGETGELFFGEGSRLTVLEDLNKVFPPEVAVFEPSKAEIAHTQKATLVCLATGFFPDHVELSWWVNGKEVHSGVSTDPQPLKEQPALNDSRYCLSSRLRVSATFWQNPRNHFRCQVQFYGLSENDEWTQDRAKPVTQIVSAEAWGRADCGITSASYHQGVLSATILYEILLGKATLYAVLVSALVLMAMVKRKDF

SEQ ID NO: 13 - DNA, 927 bp, synthetic construct
  source 1..927: mol_type = other DNA
atgggcaccagactgttcttttacgtggccctgtgcctgctgtgggccggacatagagatgccgagatcacacagagccccagacacaagatcaccgagacaggcagacaagtgaccctggcctgtcaccagacctggaaccacaacaacatgttctggtacagacaggacctcggccacggcctgagactgatccactactcttacggcgtgcacgacaccaacaagggcgaagtgtctgacggctacagcgtgtccagaagcaacaccgaggacctgcctctgacactggaatctgccgccagctctcagaccagcgtgtacttttgtgcctctagcggagccggcgaaaccggcgaactgtttttcggagagggcagcagactgaccgtgctcgaggacctgaacaaggtgttccctccggaggtggccgtgttcgagcccagcaaagccgagatcgcgcacacccagaaggccaccctggtgtgcctggccaccggcttcttccccgaccacgtggagctgagctggtgggtgaacggcaaggaggtgcacagcggcgtgagcaccgacccccagcccctgaaggagcagcccgccctgaacgacagccgctactgcctgagcagccgcctgcgcgtgagcgccaccttctggcagaacccccgcaaccacttccgctgccaggtgcagttctacggcctgagcgagaacgacgagtggacccaggaccgcgccaagcccgtgacccagatcgtgagcgccgaggcctggggccgcgccgactgcggcattaccagcgcgagctaccatcagggcgtgctgagcgccaccatcctgtacgagatcctgctgggcaaggccaccctgtacgccgtgctggtgagcgccctggtgctgatggcgatggtgaagcgcaaggacttc

SEQ ID NO: 14 - protein, 6 aa, synthetic construct
SSVSVY

SEQ ID NO: 15 - protein, 8 aa, synthetic construct
YLSGSTLV

SEQ ID NO: 16 - protein, 13 aa, synthetic construct
CAVSRSGNTPLVF

SEQ ID NO: 17 - DNA, 18 bp, synthetic construct
  source 1..18: mol_type = other DNA
agcagcgtgtccgtgtac

SEQ ID NO: 18 - DNA, 24 bp, synthetic construct
  source 1..24: mol_type = other DNA
tatctgagcggcagcaccctggtg

SEQ ID NO: 19 - DNA, 39 bp, synthetic construct
  source 1..39: mol_type = other DNA
tgcgccgtgtccagaagcggaaacacccctctggtgttc

SEQ ID NO: 20 - protein, 133 aa, synthetic construct
MLLLLVPAFQVIFTLGGTRAQSVTQLDSQVPVFEEAPVELRCNYSSSVSVYLFWYVQYPNQGLQLLLKYLSGSTLVESINGFEAEFNKSQTSFHLRKPSVHISDTAEYFCAVSRSGNTPLVFGKGTRLSVIAN

SEQ ID NO: 21 - DNA, 399 bp, synthetic construct
  source 1..399: mol_type = other DNA
atgcttctgctgctggtgcctgccttccaagtgatctttaccctcggcggcacaagagcccagagcgtgacacagctggatagccaggtgccagtgttcgaggaagcccctgtcgagctgagatgcaactacagcagcagcgtgtccgtgtacctgttttggtacgtgcagtaccccaaccagggcctgcagctgctgctcaagtatctgagcggcagcaccctggtggaatccatcaatggcttcgaggccgagttcaacaagagccagaccagcttccacctgagaaagcccagcgtgcacatcagcgataccgccgagtacttctgcgccgtgtccagaagcggaaacacccctctggtgttcggcaagggcacaagactgagcgtgatcgccaat

SEQ ID NO: 22 - protein, 140 aa, synthetic construct
IQNPDPAVYQLRDSKSSDKSVCLFTDFDSQTNVSQSKDSDVYITDKTVLDMRSMDFKSNSAVAWSNKSDFACANAFNNSIIPEDTFFPSSDVPCDVKLVEKSFETDTNLNFQNLSVIGFRILLLKVAGFNLLMTLRLWSS

SEQ ID NO: 23 - DNA, 423 bp, synthetic construct
  source 1..423: mol_type = other DNA
atccagaatccggaccccgccgtgtaccagctgcgcgacagcaagagcagcgacaagagcgtgtgcctgttcaccgacttcgacagccagaccaacgtgagccagagcaaggacagcgacgtgtacatcaccgacaagaccgtgctggacatgcgcagcatggacttcaagagcaacagcgccgtggcctggagcaacaagagcgacttcgcctgcgccaacgccttcaacaacagcatcatccccgaggacaccttcttccccagcagcgatgtgccgtgcgacgtgaagctggtggagaagagcttcgagaccgacaccaacctgaacttccagaacctgagcgtgatcggcttccgcatcctgctgctgaaggtggccggcttcaacctgctgatgaccctgcgcctgtggagcagctga

SEQ ID NO: 24 - protein, 273 aa, synthetic construct
MLLLLVPAFQVIFTLGGTRAQSVTQLDSQVPVFEEAPVELRCNYSSSVSVYLFWYVQYPNQGLQLLLKYLSGSTLVESINGFEAEFNKSQTSFHLRKPSVHISDTAEYFCAVSRSGNTPLVFGKGTRLSVIANIQNPDPAVYQLRDSKSSDKSVCLFTDFDSQTNVSQSKDSDVYITDKTVLDMRSMDFKSNSAVAWSNKSDFACANAFNNSIIPEDTFFPSSDVPCDVKLVEKSFETDTNLNFQNLSVIGFRILLLKVAGFNLLMTLRLWSS

SEQ ID NO: 25 - DNA, 819 bp, synthetic construct
  source 1..819: mol_type = other DNA
atgcttctgctgctggtgcctgccttccaagtgatctttaccctcggcggcacaagagcccagagcgtgacacagctggatagccaggtgccagtgttcgaggaagcccctgtcgagctgagatgcaactacagcagcagcgtgtccgtgtacctgttttggtacgtgcagtaccccaaccagggcctgcagctgctgctcaagtatctgagcggcagcaccctggtggaatccatcaatggcttcgaggccgagttcaacaagagccagaccagcttccacctgagaaagcccagcgtgcacatcagcgataccgccgagtacttctgcgccgtgtccagaagcggaaacacccctctggtgttcggcaagggcacaagactgagcgtgatcgccaatatccagaatccggaccccgccgtgtaccagctgcgcgacagcaagagcagcgacaagagcgtgtgcctgttcaccgacttcgacagccagaccaacgtgagccagagcaaggacagcgacgtgtacatcaccgacaagaccgtgctggacatgcgcagcatggacttcaagagcaacagcgccgtggcctggagcaacaagagcgacttcgcctgcgccaacgccttcaacaacagcatcatccccgaggacaccttcttccccagcagcgatgtgccgtgcgacgtgaagctggtggagaagagcttcgagaccgacaccaacctgaacttccagaacctgagcgtgatcggcttccgcatcctgctgctgaaggtggccggcttcaacctgctgatgaccctgcgcctgtggagcagc

SEQ ID NO: 26 - protein, 233 aa, synthetic construct
MQIPQAPWPVVWAVLQLGWRPGWFLDSPDRPWNPPTFSPALLVVTEGDNATFTCSFSNTSESFVLNWYRMSPSNQTDKLAAFPEDRSQPGQDCRFRVTQLPNGRDFHMSVVRARRNDSGTYLCGAISLAPKAQIKESLRAELRVTERRAEVPTAHPSPSPRPAGQFQTLVVGVVGGLLGSLVLLVWVLAVIKRGRKKLLYIFKQPFMRPVQTTQEEDGCSCRFPEEEEGGCEL

SEQ ID NO: 27 - DNA, 699 bp, synthetic construct
  source 1..699: mol_type = other DNA
atgcaaattcctcaagctccttggcctgtcgtgtgggccgttctgcaacttggatggcggcctggctggttcctggactctcctgacagaccctggaatcctccaacattcagccccgctctgctggtggttaccgagggcgataatgccaccttcacctgtagcttcagcaacaccagcgagagcttcgtgctgaactggtacagaatgagccccagcaaccagaccgacaagctggccgcctttcctgaggatagatctcagcccggccaggactgccggttcagagttacacagctgcccaacggccgggacttccacatgtctgtcgtccgggccagaagaaacgacagcggcacatatctgtgcggcgccatttctctggcccctaaggctcagatcaaagagagcctgagagccgagctgagagtgacagaaagacgggccgaagtgcccacagctcacccttcaccttctccaagacctgccggccagttccagacactggtcgtgggagttgttggcggactgctgggatctctggtgctgcttgtttgggtgctcgccgtgatcaagcggggcagaaagaagctgctgtacatcttcaagcagcccttcatgcggcccgtgcagaccacacaagaggaagatggctgctcctgcagattccccgaggaagaagaaggcggctgcgaactc

SEQ ID NO: 28 - protein, 170 aa, synthetic construct
MQIPQAPWPVVWAVLQLGWRPGWFLDSPDRPWNPPTFSPALLVVTEGDNATFTCSFSNTSESFVLNWYRMSPSNQTDKLAAFPEDRSQPGQDCRFRVTQLPNGRDFHMSVVRARRNDSGTYLCGAISLAPKAQIKESLRAELRVTERRAEVPTAHPSPSPRPAGQFQTLV

SEQ ID NO: 29 - DNA, 510 bp, synthetic construct
  source 1..510: mol_type = other DNA
atgcaaattcctcaagctccttggcctgtcgtgtgggccgttctgcaacttggatggcggcctggctggttcctggactctcctgacagaccctggaatcctccaacattcagccccgctctgctggtggttaccgagggcgataatgccaccttcacctgtagcttcagcaacaccagcgagagcttcgtgctgaactggtacagaatgagccccagcaaccagaccgacaagctggccgcctttcctgaggatagatctcagcccggccaggactgccggttcagagttacacagctgcccaacggccgggacttccacatgtctgtcgtccgggccagaagaaacgacagcggcacatatctgtgcggcgccatttctctggcccctaaggctcagatcaaagagagcctgagagccgagctgagagtgacagaaagacgggccgaagtgcccacagctcacccttcaccttctccaagacctgccggccagttccagacactggtc

SEQ ID NO: 30 - protein, 21 aa, synthetic construct
VGVVGGLLGSLVLLVWVLAVI

SEQ ID NO: 31 - DNA, 63 bp, synthetic construct
  source 1..63: mol_type = other DNA
gtgggagttgttggcggactgctgggatctctggtgctgcttgtttgggtgctcgccgtgatc

SEQ ID NO: 32 - protein, 42 aa, synthetic construct
KRGRKKLLYIFKQPFMRPVQTTQEEDGCSCRFPEEEEGGCEL

SEQ ID NO: 33 - DNA, 126 bp, synthetic construct
  source 1..126: mol_type = other DNA
aagcggggcagaaagaagctgctgtacatcttcaagcagcccttcatgcggcccgtgcagaccacacaagaggaagatggctgctcctgcagattccccgaggaagaagaaggcggctgcgaactc

SEQ ID NO: 34 - protein, 10 aa, synthetic construct
VVVGACGVGK

SEQ ID NO: 35 - protein, 9 aa, synthetic construct
VVGADGVGK

SEQ ID NO: 36 - protein, 9 aa, synthetic construct
VVGACGVGK

SEQ ID NO: 37 - protein, 24 aa, synthetic construct
MTEYKLVVVGAGGVGKSALTIQLI

SEQ ID NO: 38 - protein, 192 aa, synthetic construct
EDLNKVFPPEVAVFEPSKAEIAHTQKATLVCLATGFFPDHVELSWWVNGKEVHSGVSTDPQPLKEQPALNDGSGGEVPKDRFSGSGSRYCLSSRLRVSATFWQNPRNHFRCQVQFYGLSENDEWTQDRAKPVTQIVSAEAWGRADCGITSASYHQGVLSATILYEILLGKATLYAVLVSALVLMAMVKRKDF

SEQ ID NO: 39 - DNA, 576 bp, synthetic construct
  source 1..576: mol_type = other DNA
gaggacctgaacaaggtgttccctccggaggtggccgtgttcgagcccagcaaagccgagatcgcgcacacccagaaggccaccctggtgtgcctggccaccggcttcttccccgaccacgtggagctgagctggtgggtgaacggcaaggaggtgcacagcggcgtgagcaccgacccccagcccctgaaggagcagcccgccctgaacgacggatctggcggcgaagtgcccaaggacagattttccggatctggaagccgctactgcctgagcagccgcctgcgcgtgagcgccaccttctggcagaacccccgcaaccacttccgctgccaggtgcagttctacggcctgagcgagaacgacgagtggacccaggaccgcgccaagcccgtgacccagatcgtgagcgccgaggcctggggccgcgccgactgcggcattaccagcgcgagctaccatcagggcgtgctgagcgccaccatcctgtacgagatcctgctgggcaaggccaccctgtacgccgtgctggtgagcgccctggtgctgatggcgatggtgaagcgcaaggacttc

SEQ ID NO: 40 - protein, 134 aa, synthetic construct
MTEYKLVVVGADGVGKSALTIQLIQNHFVDEYDPTIEDSYRKQVVIDGETCLLDILDTAGQEEYSAMRDQYMRTGEGFLCVFAINNTKSFEDIHHYREQIKRVKDSEDVPMVLVGNKCDLPSRTVDTKQAQDLA

SEQ ID NO: 41 - protein, 15 aa, synthetic construct
GSGGEVPKDRFSGSG

SEQ ID NO: 42 - protein, 9 aa, synthetic construct
GEVPKDRFS

SEQ ID NO: 43 - protein, 12 aa, synthetic construct
GSGEVPKDRGSG

SEQ ID NO: 44 - protein, 6 aa, synthetic construct
EVPKDR

SEQ ID NO: 45 - protein, 189 aa, synthetic construct
EDLNKVFPPEVAVFEPSKAEIAHTQKATLVCLATGFFPDHVELSWWVNGKEVHSGVSTDPQPLKEQPALNDGSGEVPKDRGSGSRYCLSSRLRVSATFWQNPRNHFRCQVQFYGLSENDEWTQDRAKPVTQIVSAEAWGRADCGITSASYHQGVLSATILYEILLGKATLYAVLVSALVLMAMVKRKDF

SEQ ID NO: 46 - protein, 192 aa, synthetic construct; identical to SEQ ID NO: 38

SEQ ID NO: 47 - DNA, 567 bp, synthetic construct
  source 1..567: mol_type = other DNA
gaggacctgaacaaggtgttccctccggaggtggccgtgttcgagcccagcaaagccgagatcgcgcacacccagaaggccaccctggtgtgcctggccaccggcttcttccccgaccacgtggagctgagctggtgggtgaacggcaaggaggtgcacagcggcgtgagcaccgacccccagcccctgaaggagcagcccgccctgaacgacggatctggcgaagtgcccaaggacagaggatctggaagccgctactgcctgagcagccgcctgcgcgtgagcgccaccttctggcagaacccccgcaaccacttccgctgccaggtgcagttctacggcctgagcgagaacgacgagtggacccaggaccgcgccaagcccgtgacccagatcgtgagcgccgaggcctggggccgcgccgactgcggcattaccagcgcgagctaccatcagggcgtgctgagcgccaccatcctgtacgagatcctgctgggcaaggccaccctgtacgccgtgctggtgagcgccctggtgctgatggcgatggtgaagcgcaaggacttc

SEQ ID NO: 48 - DNA, 576 bp, synthetic construct; identical to SEQ ID NO: 39
  source 1..576: mol_type = other DNA